European Patent Application EP 4 737 483 A1, published May 6, 2026. Title: METHOD FOR PRODUCING ANTIBODY-DRUG CONJUGATE INCLUDING PURIFICATION STEP USING ACTIVATED CARBON MATERIALS. Applicant: 第一三共株式会社. Application JP. The sequence listing filed with the application follows.

SEQUENCE LISTING (17 sequences)

SEQ ID NO: 1 - protein, 472 aa, synthetic construct
  REGION 1..472: note = Heavy chain of anti-GPR20 antibody (h046-H4e)
MKHLWFFLLLVAAPRWVLSEVQLVQSGAEVKKPGASVKVSCKASGYTFTSYYISWIRQAPGQGLKYMGFINPGSGHTNYNEKFKGRVTITADKSSSTATMELSSLRSEDTAVYYCARGAGGFLRIITKFDYWGQGTLVTVSSASTKGPSVFPLAPSSKSTSGGTAALGCLVKDYFPEPVTVSWNSGALTSGVHTFPAVLQSSGLYSLSSVVTVPSSSLGTQTYICNVNHKPSNTKVDKRVEPKSCDKTHTCPPCPAPELLGGPSVFLFPPKPKDTLMISRTPEVTCVVVDVSHEDPEVKFNWYVDGVEVHNAKTKPREEQYNSTYRVVSVLTVLHQDWLNGKEYKCKVSNKALPAPIEKTISKAKGQPREPQVYTLPPSREEMTKNQVSLTCLVKGFYPSDIAVEWESNGQPENNYKTTPPVLDSDGSFFLYSKLTVDKSRWQQGNVFSCSVMHEALHNHYTQKSLSLSPGK

SEQ ID NO: 2 - protein, 234 aa, synthetic construct
  REGION 1..234: note = Light chain of anti-GPR20 antibody (h046-L7)
MVLQTQVFISLLLWISGAYGDTQLTQSPSSLSASVGDRVTITCRASKSVSTYIHWYQQKPGKQPKLLIYSAGNLESGVPSRFSGSGSGTDFTLTISSLQPEDFANYYCQQINELPYTFGQGTKVEIKRTVAAPSVFIFPPSDEQLKSGTASVVCLLNNFYPREAKVQWKVDNALQSGNSQESVTEQDSKDSTYSLSSTLTLSKADYEKHKVYACEVTHQGLSSPVTKSFNRGEC

SEQ ID NO: 3 - protein, 468 aa, synthetic construct
  REGION 1..468: note = Heavy chain of anti-CD37 antibody (hmAb-H541)
MKHLWFFLLLVAAPRWVLSEVQLVQSGAEVKKPGASVKVSCKASGYSFTDYNMYWVRQAPGQSLEWMGYIDPYNGDTTYNQKFQGRVTMTRDTSISTAYMELSRLRSDDTAVYYCARSPYGHYAMDYWGQGTTVTVSSASTKGPSVFPLAPSSKSTSGGTAALGCLVKDYFPEPVTVSWNSGALTSGVHTFPAVLQSSGLYSLSSVVTVPSSSLGTQTYICNVNHKPSNTKVDKKVEPKSCDKTHTCPPCPAPELLGGPSVFLFPPKPKDTLMISRTPEVTCVVVDVSHEDPEVKFNWYVDGVEVHNAKTKPREEQYNSTYRVVSVLTVLHQDWLNGKEYKCKVSNKALPAPIEKTISKAKGQPREPQVYTLPPSREEMTKNQVSLTCLVKGFYPSDIAVEWESNGQPENNYKTTPPVLDSDGSFFLYSKLTVDKSRWQQGNVFSCSVMHEALHNHYTQKSLSLSPGK

SEQ ID NO: 4 - protein, 234 aa, synthetic construct
  REGION 1..234: note = Light chain of anti-CD37 antibody (hmAb-L11)
MVLQTQVFISLLLWISGAYGDIQMTQSPSSLSASVGDRVTITCKASQDVSTAVDWYQQKPGKAPKLLINWASTRHTGVPSRFSGSGSGTDFTLTISSLQPEDFATYYCRQHYSTPFTFGQGTKVEIKRTVAAPSVFIFPPSDEQLKSGTASVVCLLNNFYPREAKVQWKVDNALQSGNSQESVTEQDSKDSTYSLSSTLTLSKADYEKHKVYACEVTHQGLSSPVTKSFNRGEC

SEQ ID NO: 5 - protein, 447 aa, synthetic construct
  REGION 1..447: note = Heavy chain of anti-MUC1 antibody (N54Q)
EVQLVESGGGLVQPGGSMRLSCVASGFPFSNYWMNWVRQAPGKGLEWVGEIRLKSNQYTTHYAESVKGRFTISRDDSKNSLYLQMNSLKTEDTAVYYCTRHYYFDYWGQGTLVTVSSASTKGPSVFPLAPSSKSTSGGTAALGCLVKDYFPEPVTVSWNSGALTSGVHTFPAVLQSSGLYSLSSVVTVPSSSLGTQTYICNVNHKPSNTKVDKKVEPKSCDKTHTCPPCPAPELLGGPSVFLFPPKPKDTLMISRTPEVTCVVVDVSHEDPEVKFNWYVDGVEVHNAKTKPREEQYNSTYRVVSVLTVLHQDWLNGKEYKCKVSNKALPAPIEKTISKAKGQPREPQVYTLPPSRDELTKNQVSLTCLVKGFYPSDIAVEWESNGQPENNYKTTPPVLDSDGSFFLYSKLTVDKSRWQQGNVFSCSVMHEGLHNHYTQKSLSLSPGK

SEQ ID NO: 6 - protein, 447 aa, synthetic construct
  REGION 1..447: note = Heavy chain of anti-MUC1 antibody (PankoMab)
EVQLVESGGGLVQPGGSMRLSCVASGFPFSNYWMNWVRQAPGKGLEWVGEIRLKSNNYTTHYAESVKGRFTISRDDSKNSLYLQMNSLKTEDTAVYYCTRHYYFDYWGQGTLVTVSSASTKGPSVFPLAPSSKSTSGGTAALGCLVKDYFPEPVTVSWNSGALTSGVHTFPAVLQSSGLYSLSSVVTVPSSSLGTQTYICNVNHKPSNTKVDKKVEPKSCDKTHTCPPCPAPELLGGPSVFLFPPKPKDTLMISRTPEVTCVVVDVSHEDPEVKFNWYVDGVEVHNAKTKPREEQYNSTYRVVSVLTVLHQDWLNGKEYKCKVSNKALPAPIEKTISKAKGQPREPQVYTLPPSRDELTKNQVSLTCLVKGFYPSDIAVEWESNGQPENNYKTTPPVLDSDGSFFLYSKLTVDKSRWQQGNVFSCSVMHEGLHNHYTQKSLSLSPGK

SEQ ID NO: 7 - protein, 219 aa, synthetic construct
  REGION 1..219: note = Light chain of anti-MUC1 antibody (N54Q and PankoMab)
DIVMTQSPLSNPVTPGEPASISCRSSKSLLHSNGITYFFWYLQKPGQSPQLLIYQMSNLASGVPDRFSGSGSGTDFTLRISRVEAEDVGVYYCAQNLELPPTFGQGTKVEIKRTVAAPSVFIFPPSDEQLKSGTASVVCLLNNFYPREAKVQWKVDNALQSGNSQESVTEQDSKDSTYSLSSTLTLSKADYEKHKVYACEVTHQGLSSPVTKSFNRGEC

SEQ ID NO: 8 - protein, 450 aa, synthetic construct
  REGION 1..450: note = Heavy chain of anti-HER2 antibody
EVQLVESGGGLVQPGGSLRLSCAASGFNIKDTYIHWVRQAPGKGLEWVARIYPTNGYTRYADSVKGRFTISADTSKNTAYLQMNSLRAEDTAVYYCSRWGGDGFYAMDYWGQGTLVTVSSASTKGPSVFPLAPSSKSTSGGTAALGCLVKDYFPEPVTVSWNSGALTSGVHTFPAVLQSSGLYSLSSVVTVPSSSLGTQTYICNVNHKPSNTKVDKKVEPKSCDKTHTCPPCPAPELLGGPSVFLFPPKPKDTLMISRTPEVTCVVVDVSHEDPEVKFNWYVDGVEVHNAKTKPREEQYNSTYRVVSVLTVLHQDWLNGKEYKCKVSNKALPAPIEKTISKAKGQPREPQVYTLPPSREEMTKNQVSLTCLVKGFYPSDIAVEWESNGQPENNYKTTPPVLDSDGSFFLYSKLTVDKSRWQQGNVFSCSVMHEALHNHYTQKSLSLSPGK

SEQ ID NO: 9 - protein, 214 aa, synthetic construct
  REGION 1..214: note = Light chain of anti-HER2 antibody
DIQMTQSPSSLSASVGDRVTITCRASQDVNTAVAWYQQKPGKAPKLLIYSASFLYSGVPSRFSGSRSGTDFTLTISSLQPEDFATYYCQQHYTTPPTFGQGTKVEIKRTVAAPSVFIFPPSDEQLKSGTASVVCLLNNFYPREAKVQWKVDNALQSGNSQESVTEQDSKDSTYSLSSTLTLSKADYEKHKVYACEVTHQGLSSPVTKSFNRGEC

SEQ ID NO: 10 - protein, 470 aa, synthetic construct
  REGION 1..470: note = Heavy chain of anti-TROP2 antibody (hTINA1-H1)
MKHLWFFLLLVAAPRWVLSQVQLVQSGAEVKKPGASVKVSCKASGYTFTTAGMQWVRQAPGQGLEWMGWINTHSGVPKYAEDFKGRVTISADTSTSTAYLQLSSLKSEDTAVYYCARSGFGSSYWYFDVWGQGTLVTVSSASTKGPSVFPLAPSSKSTSGGTAALGCLVKDYFPEPVTVSWNSGALTSGVHTFPAVLQSSGLYSLSSVVTVPSSSLGTQTYICNVNHKPSNTKVDKRVEPKSCDKTHTCPPCPAPELLGGPSVFLFPPKPKDTLMISRTPEVTCVVVDVSHEDPEVKFNWYVDGVEVHNAKTKPREEQYNSTYRVVSVLTVLHQDWLNGKEYKCKVSNKALPAPIEKTISKAKGQPREPQVYTLPPSREEMTKNQVSLTCLVKGFYPSDIAVEWESNGQPENNYKTTPPVLDSDGSFFLYSKLTVDKSRWQQGNVFSCSVMHEALHNHYTQKSLSLSPGK

SEQ ID NO: 11 - protein, 234 aa, synthetic construct
  REGION 1..234: note = Light chain of anti-TROP2 antibody (hTINA1-L1)
MVLQTQVFISLLLWISGAYGDIQMTQSPSSLSASVGDRVTITCKASQDVSTAVAWYQQKPGKAPKLLIYSASYRYTGVPSRFSGSGSGTDFTLTISSLQPEDFAVYYCQQHYITPLTFGQGTKLEIKRTVAAPSVFIFPPSDEQLKSGTASVVCLLNNFYPREAKVQWKVDNALQSGNSQESVTEQDSKDSTYSLSSTLTLSKADYEKHKVYACEVTHQGLSSPVTKSFNRGEC

SEQ ID NO: 12 - protein, 447 aa, synthetic construct
  REGION 1..447: note = Heavy chain of anti-HER3 antibody
QVQLQQWGAGLLKPSETLSLTCAVYGGSFSGYYWSWIRQPPGKGLEWIGEINHSGSTNYNPSLKSRVTISVETSKNQFSLKLSSVTAADTAVYYCARDKWTWYFDLWGRGTLVTVSSASTKGPSVFPLAPSSKSTSGGTAALGCLVKDYFPEPVTVSWNSGALTSGVHTFPAVLQSSGLYSLSSVVTVPSSSLGTQTYICNVNHKPSNTKVDKRVEPKSCDKTHTCPPCPAPELLGGPSVFLFPPKPKDTLMISRTPEVTCVVVDVSHEDPEVKFNWYVDGVEVHNAKTKPREEQYNSTYRVVSVLTVLHQDWLNGKEYKCKVSNKALPAPIEKTISKAKGQPREPQVYTLPPSREEMTKNQVSLTCLVKGFYPSDIAVEWESNGQPENNYKTTPPVLDSDGSFFLYSKLTVDKSRWQQGNVFSCSVMHEALHNHYTQKSLSLSPGK

SEQ ID NO: 13 - protein, 220 aa, synthetic construct
  REGION 1..220: note = Light chain of anti-HER3 antibody
DIEMTQSPDSLAVSLGERATINCRSSQSVLYSSSNRNYLAWYQQNPGQPPKLLIYWASTRESGVPDRFSGSGSGTDFTLTISSLQAEDVAVYYCQQYYSTPRTFGQGTKVEIKRTVAAPSVFIFPPSDEQLKSGTASVVCLLNNFYPREAKVQWKVDNALQSGNSQESVTEQDSKDSTYSLSSTLTLSKADYEKHKVYACEVTHQGLSSPVTKSFNRGEC

SEQ ID NO: 14 - protein, 471 aa, synthetic construct
  REGION 1..471: note = Heavy chain of anti-B7-H3 antibody (M30-H1)
MKHLWFFLLLVAAPRWVLSQVQLVQSGAEVKKPGSSVKVSCKASGYTFTNYVMHWVRQAPGQGLEWMGYINPYNDDVKYNEKFKGRVTITADESTSTAYMELSSLRSEDTAVYYCARWGYYGSPLYYFDYWGQGTLVTVSSASTKGPSVFPLAPSSKSTSGGTAALGCLVKDYFPEPVTVSWNSGALTSGVHTFPAVLQSSGLYSLSSVVTVPSSSLGTQTYICNVNHKPSNTKVDKRVEPKSCDKTHTCPPCPAPELLGGPSVFLFPPKPKDTLMISRTPEVTCVVVDVSHEDPEVKFNWYVDGVEVHNAKTKPREEQYNSTYRVVSVLTVLHQDWLNGKEYKCKVSNKALPAPIEKTISKAKGQPREPQVYTLPPSREEMTKNQVSLTCLVKGFYPSDIAVEWESNGQPENNYKTTPPVLDSDGSFFLYSKLTVDKSRWQQGNVFSCSVMHEALHNHYTQKSLSLSPGK

SEQ ID NO: 15 - protein, 233 aa, synthetic construct
  REGION 1..233: note = Light chain of anti-B7-H3 antibody (M30-L4)
MVLQTQVFISLLLWISGAYGEIVLTQSPATLSLSPGERATLSCRASSRLIYMHWYQQKPGQAPRPLIYATSNLASGIPARFSGSGSGTDFTLTISSLEPEDFAVYYCQQWNSNPPTFGQGTKVEIKRTVAAPSVFIFPPSDEQLKSGTASVVCLLNNFYPREAKVQWKVDNALQSGNSQESVTEQDSKDSTYSLSSTLTLSKADYEKHKVYACEVTHQGLSSPVTKSFNRGEC

SEQ ID NO: 16 - protein, 471 aa, synthetic construct
  REGION 1..471: note = Heavy chain of anti-CDH6 antibody (hH01)
MKHLWFFLLLVAAPRWVLSEVQLVQSGAEVKKPGASVKVSCKASGYTFTRNFMHWVRQAPGQGLEWMGWIYPGDGETEYAQKFQGRVTITADTSTSTAYMELSSLRSEDTAVYYCARGVYGGFAGGYFDFWGQGTLVTVSSASTKGPSVFPLAPSSKSTSGGTAALGCLVKDYFPEPVTVSWNSGALTSGVHTFPAVLQSSGLYSLSSVVTVPSSSLGTQTYICNVNHKPSNTKVDKRVEPKSCDKTHTCPPCPAPELLGGPSVFLFPPKPKDTLMISRTPEVTCVVVDVSHEDPEVKFNWYVDGVEVHNAKTKPREEQYNSTYRVVSVLTVLHQDWLNGKEYKCKVSNKALPAPIEKTISKAKGQPREPQVYTLPPSREEMTKNQVSLTCLVKGFYPSDIAVEWESNGQPENNYKTTPPVLDSDGSFFLYSKLTVDKSRWQQGNVFSCSVMHEALHNHYTQKSLSLSPGK

SEQ ID NO: 17 - protein, 233 aa, synthetic construct
  REGION 1..233: note = Light chain of anti-CDH6 antibody (hL02)
MVLQTQVFISLLLWISGAYGDIQMTQSPSSLSASVGDRVTITCKASQNIYKNLAWYQQKPGKAPKLLIYDANTLQTGVPSRFSGSGSGSDFTLTISSLQPEDFATYFCQQYYSGWAFGQGTKVEIKRTVAAPSVFIFPPSDEQLKSGTASVVCLLNNFYPREAKVQWKVDNALQSGNSQESVTEQDSKDSTYSLSSTLTLSKADYEKHKVYACEVTHQGLSSPVTKSFNRGEC